European Patent Specification EP 3 218 517 B1, published May 1, 2024. Title: MiR-214 as a diagnostic and prognostic biomarker specific for ulcerative colitis and a miR-214 inhibitor for treatment of same. Applicant: The Regents of the University of California. The sequence listing filed with the application follows.

SEQUENCE LISTING (14 sequences)

SEQ ID NO: 1 - DNA, 15 bp, Artificial
  synthetic inhibitor of microRNA
tgtctgtgcctgctg

SEQ ID NO: 2 - skipped

SEQ ID NO: 3 - RNA, 22 nt, Homo sapiens
ugagacacugcauuccugcugg

SEQ ID NO: 4 - RNA, 22 nt, Homo sapiens
uuucaaucauaauaccugcugu

SEQ ID NO: 5 - DNA, 19 bp, Artificial
  Primer
cccagacatgacagccatc

SEQ ID NO: 6 - DNA, 20 bp, Artificial
  Primer
tctgcaggaaatcccatagc

SEQ ID NO: 7 - DNA, 20 bp, Artificial
  Primer
atggccacgattatgtctcc

SEQ ID NO: 8 - DNA, 20 bp, Artificial
  Primer
gcccatcatggtgactaagg

SEQ ID NO: 9 - DNA, 20 bp, Artificial
  Primer
cccagcacaatgaagatcaa

SEQ ID NO: 10 - DNA, 20 bp, Artificial
  Primer
acatctgctggaaggtggac

SEQ ID NO: 11 - DNA, 20 bp, Artificial
  Primer
atgttcgtcatgggtgtgaa

SEQ ID NO: 12 - DNA, 20 bp, Artificial
  Primer
ggtgctaagcagttggtggt

SEQ ID NO: 13 - DNA, 20 bp, Artificial
  Primer
gggcttgagtccatcagctt

SEQ ID NO: 14 - DNA, 20 bp, Artificial
  Primer
gttcagcaggacaggtctca